European Patent Application EP 4 163 377 A1, published April 12, 2023. Title: RECOMBINANT STRAIN FOR PRODUCING L-AMINO ACID, CONSTRUCTION METHOD THEREFOR, AND APPLICATION THEREOF. Applicant: INNER MONGOLIA EPPEN BIOTECH CO., LTD. The sequence listing filed with the application follows.

SEQUENCE LISTING (64 sequences)

SEQ ID NO: 1 - DNA, 1083 bp, Corynebacterium glutamicum
gtgtcacacaccgcgtccacaccgacgccagaggaatactccgcgcagcaacccagcacccagggcactcgcgttgagttccgcggcataaccaaagtctttagcaacaataaatctgctaaaaccaccgcgcttgataatgtcactctcaccgtagaacccggtgaggtaatcggcatcatcggttactctggcgccggcaagtccactcttgtccgcctcatcaatggccttgactcccccacgagcggttcgttgctgctcaacggcaccgacatcgtcggaatgcccgagtctaagctgcgtaaactgcgcagtaatatcggcatgattttccagcagttcaacctgttccagtcgcgtactgcggctggaaatgtggagtacccgctggaagttgccaagatggacaaggcagctcgtaaagctcgcgtgcaagaaatgctcgagttcgtcggcctgggcgacaaaggcaaaaactaccccgagcagctgtcgggcggccagaagcagcgcgtcggcattgcccgtgcactggccaccaatccaacgcttttgcttgccgacgaagccacctccgctttggacccagaaaccacccatgaagttctggagctgctgcgcaaggtaaaccgcgaactgggcatcaccatcgttgtgatcacccacgaaatggaagttgtgcgttccatcgcagacaaggttgctgtgatggaatccggcaaagttgtggaatacggcagcgtctacgaggtgttctccaatccacaaacacaggttgctcaaaagttcgtggccaccgcgctgcgtaacaccccagaccaagtggaatcggaagatctgcttagccatgagggacgtctgttcaccattgatctgactgaaacgtccggcttctttgcagcaaccgctcgtgctgccgaacaaggtgcttttgtcaacatcgttcacggtggcgtgaccaccttgcaacgccaatcatttggcaaaatgactgttcgactcaccggcaacaccgctgcgattgaagagttctatcaaaccttgaccaagaccacgaccatcaaggagatcacccgatga

SEQ ID NO: 2 - DNA, 1083 bp, artifical sequence
gtgtcacacaccgcgtccacaccgacgccagaggaatactccgcgcagcaacccagcacccagggcactcgcgttgagttccgcggcataaccaaagtctttagcaacaataaatctgctaaaaccaccgcgcttgataatgtcactctcaccgtagaacccggtgaggtaatcggcatcatcggttactctggcgccggcaagtccactcttgtccgcctcatcaatggccttgactcccccacgagcggttcgttgctgctcaacggcaccgacatcgtcggaatgcccgagtctaagctgcgtaaactgcgcagtaatatcggcatgattttccagcagttcaacctgttccagtcgcgtactgcggctggaaatgtggagtacccgctggaagttgccaagatggacaaggcagctcgtaaagctcgcgtgcaagaaatgctcgagttcgtcggcctgggcgacaaaggcaaaaactaccccgagcagctgtcgggcggccagaagcagcgcgtcggcattgcccgtgcactggccaccaatccaacgcttttgcttgccgacgaagccacctccgctttggacccagaaaccacccatgaagttctggagctgctgcgcaaggtaaaccgcgaactgggcatcaccatcgttgtgatcacccacgaaatggaagttgtgcgttccatcgcagacaaggttgctgtgatggaatccggcaaagttgtggaatacggcagcgtctacgaggtgttctccaatccacaaacacaggttgctcaaaagttcgtggccaccgcgctgcgtaacaccccagaccaagtggaatcggaagatctgcttagccatgagggacgtctgttcaccattgatctgactgaaacgtccggcttctttgcagcaaccgctcgtgctgccgaacaaggtgcttttgtcaacatcgttcacggtggcgtgaccaccttgcaacgccaatcatttggcaaaatgactgtttgactcaccggcaacaccgctgcgattgaagagttctatcaaaccttgaccaagaccacgaccatcaaggagatcacccgatga

SEQ ID NO: 3 - protein, 360 aa, Corynebacterium glutamicum
MSHTASTPTPEEYSAQQPSTQGTRVEFRGITKVFSNNKSAKTTALDNVTLTVEPGEVIGIIGYSGAGKSTLVRLINGLDSPTSGSLLLNGTDIVGMPESKLRKLRSNIGMIFQQFNLFQSRTAAGNVEYPLEVAKMDKAARKARVQEMLEFVGLGDKGKNYPEQLSGGQKQRVGIARALATNPTLLLADEATSALDPETTHEVLELLRKVNRELGITIVVITHEMEVVRSIADKVAVMESGKVVEYGSVYEVFSNPQTQVAQKFVATALRNTPDQVESEDLLSHEGRLFTIDLTETSGFFAATARAAEQGAFVNIVHGGVTTLQRQSFGKMTVRLTGNTAAIEEFYQTLTKTTTIKEITR

SEQ ID NO: 4 - protein, 333 aa, artifical sequence
MSHTASTPTPEEYSAQQPSTQGTRVEFRGITKVFSNNKSAKTTALDNVTLTVEPGEVIGIIGYSGAGKSTLVRLINGLDSPTSGSLLLNGTDIVGMPESKLRKLRSNIGMIFQQFNLFQSRTAAGNVEYPLEVAKMDKAARKARVQEMLEFVGLGDKGKNYPEQLSGGQKQRVGIARALATNPTLLLADEATSALDPETTHEVLELLRKVNRELGITIVVITHEMEVVRSIADKVAVMESGKVVEYGSVYEVFSNPQTQVAQKFVATALRNTPDQVESEDLLSHEGRLFTIDLTETSGFFAATARAAEQGAFVNIVHGGVTTLQRQSFGKMTV

SEQ ID NO: 5 - DNA, 55 bp, artifical sequence
cagtgccaagcttgcatgcctgcaggtcgactctagggacggcaacgtacataac

SEQ ID NO: 6 - DNA, 29 bp, artifical sequence
gttgccggtgagtcaaacagtcattttgc

SEQ ID NO: 7 - DNA, 29 bp, artifical sequence
gcaaaatgactgtttgactcaccggcaac

SEQ ID NO: 8 - DNA, 56 bp, artifical sequence
cagctatgaccatgattacgaattcgagctcggtacccgcggctggaaatgtggag

SEQ ID NO: 9 - DNA, 18 bp, artifical sequence
ctagccggttccagtcag

SEQ ID NO: 10 - DNA, 19 bp, artifical sequence
ggacgtctgttcaccattg

SEQ ID NO: 11 - DNA, 55 bp, artifical sequence
cagtgccaagcttgcatgcctgcaggtcgactctagaatgcgttctggactgagg

SEQ ID NO: 12 - DNA, 55 bp, artifical sequence; identical to SEQ ID NO: 11

SEQ ID NO: 13 - DNA, 37 bp, artifical sequence
catctgttctcggtgcaccagctgcgaggatcatctc

SEQ ID NO: 14 - DNA, 46 bp, artifical sequence
gatttaattgcgccatctgattctggcaacaactccttccttgacc

SEQ ID NO: 15 - DNA, 49 bp, artifical sequence
ggtcaaggaaggagttgttgccagaatcagatggcgcaattaaatcaag

SEQ ID NO: 16 - DNA, 60 bp, artifical sequence
cagctatgaccatgattacgaattcgagctcggtacccgctatgacaccttcaacggatc

SEQ ID NO: 17 - DNA, 19 bp, artifical sequence
tccaaggaagatacacgcc

SEQ ID NO: 18 - DNA, 18 bp, artifical sequence
cgaaatggaagttgtgcg

SEQ ID NO: 19 - DNA, 19 bp, artifical sequence
cgatgatgccgattacctc

SEQ ID NO: 20 - DNA, 18 bp, artifical sequence
cgttggaatcttgcgttg

SEQ ID NO: 21 - DNA, 55 bp, artifical sequence
gcttgcatgcctgcaggtcgactctagaggatcccccagctgcgaggatcatctc

SEQ ID NO: 22 - DNA, 54 bp, artifical sequence
atcaggctgaaaatcttctctcatccgccaaaaccaacaactccttccttgacc

SEQ ID NO: 23 - DNA, 54 bp, artifical sequence
cagtgccaagcttgcatgcctgcaggtcgactctagaatgaatgggatgggtcg

SEQ ID NO: 24 - DNA, 37 bp, artifical sequence
catcatcggttactctggccgaaatggaagttgtgcg

SEQ ID NO: 25 - DNA, 37 bp, artifical sequence
cgcacaacttccatttcggccagagtaaccgatgatg

SEQ ID NO: 26 - DNA, 58 bp, artifical sequence
cagctatgaccatgattacgaattcgagctcggtaccccaacaactccttccttgacc

SEQ ID NO: 27 - DNA, 18 bp, artifical sequence
aatgaatgggatgggtcg

SEQ ID NO: 28 - DNA, 20 bp, artifical sequence
caacaactccttccttgacc

SEQ ID NO: 29 - DNA, 2679 bp, Corynebacterium glutamicum
atggcagaatcaaacgctatggaccgggcacaaatctctgcactgctagatagagcacagcacacaatcaaccttgccgaacaagcaaacaacgtgctccgactgttgaaaacacccggaacggccacagtaggggacaacgggacactcggcaccgatacctatctgatcccatcccgcaacatcacctggcctgacaacctgtatgtcaacgtctttctagacggcatgaatgcagaagccacccttaccgattacgtcgcatcagtcgcttcgatcccacgcctatgccagatcatcaacgagggccaaggcggcatgttccgcagactattcaaccccaccaaggtccaagccggcgaccaagctgtcttcgacctcatggtcaaactcgacgagatttcatctaccacccacgaagtctcccgcatgctcgagggcgtccacgctgcccgcacccgccaacaacaaggcgttgcacttttcccaggtattcatggagtgggagagcgctacatcgaacgcgcacaacaggtactcgcctcagccctcggtatcgctggattcggtgccgaaccctgggacggacatacccttgcccaagcgcgccgggtagtccaacgctacgcccaagatcctaactccgaataccggctgaaaagcgaagccgagaaacacctcacatccatcaacgagctccgcgtacagatactcctcgaacaactccccgttgatgccctacgcatggctaccgaccaccgcctgcgctttggatccctcgattccatccacgtcgcaaccgtcgccgacgtcctaaaaacacacacctccatcctcaccaccgtgcaaggtatcggcgcccaaaccgcggggcggatgaaagccgcagcagaaacactcaaacaagaagcactacgccgccaaaacacctccatcggcgacgaacctacccaacccgccatgcgtctaatcaacgtgctggcccgcttcgaccaaaccgaaaccatcacgcccgaagaacgcgcccgccgcacccgcgtcatcgactacgtagaacacatacccccaagcctcgacccctacatcgtcatcaacccagcaacgcctgagttcaacaacttcaccgacgacctccgctggatcgacgcaaaccccaacctcttccacccacaaacaatcaccaccccacccgccgacatctgggacgactacatctcccgtcccgctcactaccaaggcctgctagccacgctgctcggccgcgacatcgaaggcgcagacgaactcctcgacgccaccaccctccaaaaaatcagagacctcaccctcgacaaaactcatctcaccgacctccacctccgcggataccaatcattcggcgcccgcttcgccatcatccaaaagaaaaccctcctcggcgacgacatgggactcggcaaaacagtccaagccctctccgcagctgcacaccttgccgccaccgaaaaagacttccgcaccctcgtcgtcgtacccgcatccgtcattgttaactggacccgcgaatgcaaacgcttcctcaacctccccgtattcatcgcccacggagacaacaaacaagacgccatcaacgcctggtctaacaccaacggaatcgcaatctgcacctacgacggcgtccgcaccatggacatccccgcgccgggtctggtcattgccgatgaagcccacctgatcaaaaacccctccaccaaacgcacccaagcactgcgcaaacttatcgacgccgccccatacacccttctgatgaccggcacaccactagaaaacaaagtggaagagtttgtaaatctcgtgcgctacatccaaccggagctgatcacccgtggcatgtccaaaatgcaggccgagaatttccgcgagcgcatcgcaccagcctatctgcgcagaaatcaagctgatgtgcttgacgaactcccagagcgcaccgactccatcgactggatcgacctcaccccagaagaccgcagcgcctacgacgaccaagtccgccaaggcagctggatgggcatgcgccgctccgccatgctctcaccaacaccacgcctaacttccgcaaaaatgcaacgcatcctagaactcttcgaagaagcagaagaacacggccgcaaagccctcatcttcacctacttcctcgacgtcctcgacgaactggaaaagcatctaggcgagcgcgtcatcggccgcatttccggcgacgtgccagccaccaagcgccaattgcttgtcgacgccctgtcccactccaaacccggatccgccctcattgcccaaatcaccgccgggggagtaggcctaaacatccaatccgcgagcctatgcattatttgtgaacctcaagtaaagccaaccatcgaacagcaggccgtcgcccgagtccaccgcatgggccaaaccgccaccgtccaagtccaccgactcatcggcgacgaaaccgcagacgaacgcatgctagaaatcctggcaggcaaaactcacgtcttcgacgtctacgcccggctatctgaaaccgcagagattccagatgctgtggatatcactgaatcacagctggcagcacgggttattgatgaggagcgtgcacggttagggcttactgaatccactggccctaaagatgaagaaacggccttaagctag

SEQ ID NO: 30 - DNA, 2679 bp, Artificial Sequence
  artifical sequence
atggcagaatcaaacgctatggaccgggcacaaatctctgcactgctagatagagcacagcacacaatcaaccttgccgaacaagcaaacaacgtgctccgactgttgaaaacacccggaacggccacagtaggggacaacgggacactcggcaccgatacctatctgatcccatcccgcaacatcacctggcctgacaacctgtatgtcaacgtctttctagacggcatgaatgcagaagccacccttaccgattacgtcgcatcagtcgcttcgatcccacgcctatgccagatcatcaacgagggccaaggcggcatgttccgcagactattcaaccccaccaaggtccaagccggcgaccaagctgtcttcgacctcatggtcaaactcgacgagatttcatctaccacccacgaagtctcccgcatgctcgagggcgtccacgctgcccgcacccgccaacaacaaggcgttgcacttttcccaggtattcatggagtgggagagcgctacatcgaacgcgcacaacaggtactcgcctcagccctcggtatcgctggattcggtgccgaaccctgggacggacatacccttgcccaagcgcgccgggtagtccaacgctacgcccaagatcctaactccgaataccggctgaaaagcgaagccgagaaacacctcacatccatcaacgagctccgcgtacagatactcctcgaacaactccccgttgatgccctacgcatggctaccgaccaccgcctgcgctttggatccctcgattccatccacgtcgcaaccgtcgccgacgtcctaaaaacacacacctccatcctcaccaccgtgcaaggtatcggcgcccaaaccgcggggcggatgaaagccgcagcagaaacactcaaacaagaagcactacgccgccaaaacacctccatcggcgacgaacctacccaacccgccatgcgtctaatcaacgtgctggcccgcttcgaccaaaccgaaaccatcacgcccgaagaacgcgcccgccgcacccgcgtcatcgactacgtagaacacatacccccaagcctcgacccctacatcgtcatcaacccagcaacgcctgagttcaacaacttcaccgacgacctccgctggatcgacgcaaaccccaacctcttccacccacaaacaatcaccaccccacccgccgacatctgggacgactacatctcccgtcccgctcactaccaaggcctgctagccacgctgctcggccgcgacatcgaaggcgcagacgaactcctcgacgccaccaccctccaaaaaatcagagacctcaccctcgacaaaactcatctcaccgacctccacctccgcggataccaatcattcggcgcccgcttcgccatcatccaaaagaaaaccctcctcggcgacgacatgggactcggcaaaacagtccaagccctctccgcagctgcacaccttgccgccaccgaaaaagacttccgcaccctcgtcgtcgtacccgcatccgtcattgttaactggacccgcgaatgcaaacgcttcctcaacctccccgtattcatcgcccacggagacaacaaacaagacgccatcaacgcctggtctaacaccaacggaatcgcaatctgcacctacgacggcgtccgcaccatggacatccccgcgccgggtctggtcattgccgatgaagcccacctgatcaaaaacccctccaccaaacgcacccaagcactgcgcaaacttatcgacgccgccccattcacccttctgatgaccggcacaccactagaaaacaaagtggaagagtttgtaaatctcgtgcgctacatccaaccggagctgatcacccgtggcatgtccaaaatgcaggccgagaatttccgcgagcgcatcgcaccagcctatctgcgcagaaatcaagctgatgtgcttgacgaactcccagagcgcaccgactccatcgactggatcgacctcaccccagaagaccgcagcgcctacgacgaccaagtccgccaaggcagctggatgggcatgcgccgctccgccatgctctcaccaacaccacgcctaacttccgcaaaaatgcaacgcatcctagaactcttcgaagaagcagaagaacacggccgcaaagccctcatcttcacctacttcctcgacgtcctcgacgaactggaaaagcatctaggcgagcgcgtcatcggccgcatttccggcgacgtgccagccaccaagcgccaattgcttgtcgacgccctgtcccactccaaacccggatccgccctcattgcccaaatcaccgccgggggagtaggcctaaacatccaatccgcgagcctatgcattatttgtgaacctcaagtaaagccaaccatcgaacagcaggccgtcgcccgagtccaccgcatgggccaaaccgccaccgtccaagtccaccgactcatcggcgacgaaaccgcagacgaacgcatgctagaaatcctggcaggcaaaactcacgtcttcgacgtctacgcccggctatctgaaaccgcagagattccagatgctgtggatatcactgaatcacagctggcagcacgggttattgatgaggagcgtgcacggttagggcttactgaatccactggccctaaagatgaagaaacggccttaagctag

SEQ ID NO: 31 - protein, 892 aa, Corynebacterium glutamicum
MAESNAMDRAQISALLDRAQHTINLAEQANNVLRLLKTPGTATVGDNGTLGTDTYLIPSRNITWPDNLYVNVFLDGMNAEATLTDYVASVASIPRLCQIINEGQGGMFRRLFNPTKVQAGDQAVFDLMVKLDEISSTTHEVSRMLEGVHAARTRQQQGVALFPGIHGVGERYIERAQQVLASALGIAGFGAEPWDGHTLAQARRVVQRYAQDPNSEYRLKSEAEKHLTSINELRVQILLEQLPVDALRMATDHRLRFGSLDSIHVATVADVLKTHTSILTTVQGIGAQTAGRMKAAAETLKQEALRRQNTSIGDEPTQPAMRLINVLARFDQTETITPEERARRTRVIDYVEHIPPSLDPYIVINPATPEFNNFTDDLRWIDANPNLFHPQTITTPPADIWDDYISRPAHYQGLLATLLGRDIEGADELLDATTLQKIRDLTLDKTHLTDLHLRGYQSFGARFAIIQKKTLLGDDMGLGKTVQALSAAAHLAATEKDFRTLVVVPASVIVNWTRECKRFLNLPVFIAHGDNKQDAINAWSNTNGIAICTYDGVRTMDIPAPGLVIADEAHLIKNPSTKRTQALRKLIDAAPYTLLMTGTPLENKVEEFVNLVRYIQPELITRGMSKMQAENFRERIAPAYLRRNQADVLDELPERTDSIDWIDLTPEDRSAYDDQVRQGSWMGMRRSAMLSPTPRLTSAKMQRILELFEEAEEHGRKALIFTYFLDVLDELEKHLGERVIGRISGDVPATKRQLLVDALSHSKPGSALIAQITAGGVGLNIQSASLCIICEPQVKPTIEQQAVARVHRMGQTATVQVHRLIGDETADERMLEILAGKTHVFDVYARLSETAEIPDAVDITESQLAARVIDEERARLGLTESTGPKDEETALS

SEQ ID NO: 32 - protein, 892 aa, Artificial Sequence
  artifical sequence
MAESNAMDRAQISALLDRAQHTINLAEQANNVLRLLKTPGTATVGDNGTLGTDTYLIPSRNITWPDNLYVNVFLDGMNAEATLTDYVASVASIPRLCQIINEGQGGMFRRLFNPTKVQAGDQAVFDLMVKLDEISSTTHEVSRMLEGVHAARTRQQQGVALFPGIHGVGERYIERAQQVLASALGIAGFGAEPWDGHTLAQARRVVQRYAQDPNSEYRLKSEAEKHLTSINELRVQILLEQLPVDALRMATDHRLRFGSLDSIHVATVADVLKTHTSILTTVQGIGAQTAGRMKAAAETLKQEALRRQNTSIGDEPTQPAMRLINVLARFDQTETITPEERARRTRVIDYVEHIPPSLDPYIVINPATPEFNNFTDDLRWIDANPNLFHPQTITTPPADIWDDYISRPAHYQGLLATLLGRDIEGADELLDATTLQKIRDLTLDKTHLTDLHLRGYQSFGARFAIIQKKTLLGDDMGLGKTVQALSAAAHLAATEKDFRTLVVVPASVIVNWTRECKRFLNLPVFIAHGDNKQDAINAWSNTNGIAICTYDGVRTMDIPAPGLVIADEAHLIKNPSTKRTQALRKLIDAAPFTLLMTGTPLENKVEEFVNLVRYIQPELITRGMSKMQAENFRERIAPAYLRRNQADVLDELPERTDSIDWIDLTPEDRSAYDDQVRQGSWMGMRRSAMLSPTPRLTSAKMQRILELFEEAEEHGRKALIFTYFLDVLDELEKHLGERVIGRISGDVPATKRQLLVDALSHSKPGSALIAQITAGGVGLNIQSASLCIICEPQVKPTIEQQAVARVHRMGQTATVQVHRLIGDETADERMLEILAGKTHVFDVYARLSETAEIPDAVDITESQLAARVIDEERARLGLTESTGPKDEETALS

SEQ ID NO: 33 - DNA, 56 bp, Artificial Sequence
  artifical sequence
cagtgccaagcttgcatgcctgcaggtcgactctagtgcgttcgtctgcggtttcg

SEQ ID NO: 34 - DNA, 30 bp, Artificial Sequence
  artifical sequence
atcgacgccgccccattcacccttctgatg

SEQ ID NO: 35 - DNA, 30 bp, Artificial Sequence
  artifical sequence
catcagaagggtgaatggggcggcgtcgat

SEQ ID NO: 36 - DNA, 57 bp, Artificial Sequence
  artifical sequence
cagctatgaccatgattacgaattcgagctcggtacccaagcctcgacccctacatc

SEQ ID NO: 37 - DNA, 20 bp, Artificial Sequence
  artifical sequence
cacatcagcttgatttctgc

SEQ ID NO: 38 - DNA, 20 bp, Artificial Sequence
  artifical sequence
ggtcattgccgatgaagccc

SEQ ID NO: 39 - DNA, 55 bp, Artificial Sequence; identical to SEQ ID NO: 11
  artifical sequence

SEQ ID NO: 40 - DNA, 36 bp, Artificial Sequence
  artifical sequence
gaaacggccttaagctaggtgcaccgagaacagatg

SEQ ID NO: 41 - DNA, 36 bp, Artificial Sequence
  artifical sequence
catctgttctcggtgcacctagcttaaggccgtttc

SEQ ID NO: 42 - DNA, 39 bp, Artificial Sequence
  artifical sequence
cttgatttaattgcgccatcaagcttttcccgcccggtt

SEQ ID NO: 43 - DNA, 39 bp, Artificial Sequence
  artifical sequence
aaccgggcgggaaaagcttgatggcgcaattaaatcaag

SEQ ID NO: 44 - DNA, 60 bp, Artificial Sequence; identical to SEQ ID NO: 16
  artifical sequence

SEQ ID NO: 45 - DNA, 19 bp, Artificial Sequence
  artifical sequence
tccaaggaagatacacgcc

SEQ ID NO: 46 - DNA, 20 bp, Artificial Sequence
  artifical sequence
cttctgatgaccggcacacc

SEQ ID NO: 47 - DNA, 20 bp, Artificial Sequence
  artifical sequence
tagtcgatgacgcgggtgcg

SEQ ID NO: 48 - DNA, 18 bp, Artificial Sequence
  artifical sequence
cgttggaatcttgcgttg

SEQ ID NO: 49 - DNA, 54 bp, Artificial Sequence
  artifical sequence
gcttgcatgcctgcaggtcgactctagaggatccccctagcttaaggccgtttc

SEQ ID NO: 50 - DNA, 53 bp, Artificial Sequence
  artifical sequence
atcaggctgaaaatcttctctcatccgccaaaacaagcttttcccgcccggtt

SEQ ID NO: 51 - DNA, 56 bp, Artificial Sequence
  artifical sequence
cagtgccaagcttgcatgcctgcaggtcgactctagaccggcgcagatgccaacgc

SEQ ID NO: 52 - DNA, 37 bp, Artificial Sequence
  artifical sequence
cccagaactgaaggtctaattgcctaaggccggaatt

SEQ ID NO: 53 - DNA, 37 bp, Artificial Sequence
  artifical sequence
aattccggccttaggcaattagaccttcagttctggg

SEQ ID NO: 54 - DNA, 56 bp, Artificial Sequence
  artifical sequence
cagctatgaccatgattacgaattcgagctcggtacccgcttgatgaaggctccag

SEQ ID NO: 55 - DNA, 20 bp, Artificial Sequence
  artifical sequence
accggcgcagatgccaacgc

SEQ ID NO: 56 - DNA, 18 bp, Artificial Sequence
  artifical sequence
gcttgatgaaggctccag

SEQ ID NO: 57 - DNA, 242 bp, Corynebacterium glutamicum
ttcagggtagttgactaaagagttgctcgcgaagtagcacctgtcacttttgtctcaaatattaaatcgaatatcaatatatggtctgtttattggaacgcgtcccagtggctgagacgcatccgctaaagccccaggaaccctgtgcagaaagaaaacactcctctggctaggtagacacagtttataaaggtagagttgagcgggtaactgtcagcacgtagatcgaaaggtgcacaaag

SEQ ID NO: 58 - DNA, 242 bp, Artificial Sequence
  artifical sequence
ttcagggtagttgactaaagagttgctcgcgaagtagcacctgtcacttttgtctcaaatattaaatcgaatatcaatatatggtctgtttattggaacgcgtcccagtggctgagacgcatccgctaaagccccaggaaccctgtgcagaaagaaaacactcctctggctaggtagacacagtttataaaggtataattgagcgggtaactgtcagcacgtagatcgaaaggtgcacaaag

SEQ ID NO: 59 - DNA, 29 bp, Artificial Sequence
  artifical sequence
ccggaattcgaccaaggatgagggctttg

SEQ ID NO: 60 - DNA, 30 bp, Artificial Sequence
  artifical sequence
agttacccgctcaattatacctttataaac

SEQ ID NO: 61 - DNA, 30 bp, Artificial Sequence
  artifical sequence
gtttataaaggtataattgagcgggtaact

SEQ ID NO: 62 - DNA, 30 bp, Artificial Sequence
  artifical sequence
acatgcatgcgcgtacgcgaagtggcacat

SEQ ID NO: 63 - DNA, 20 bp, Artificial Sequence
  artifical sequence
atcaatatatggtctgttta

SEQ ID NO: 64 - DNA, 20 bp, Artificial Sequence
  artifical sequence
cttggtggcaacgatccgtt